European Patent Specification EP 3 620 472 B1, published January 14, 2026. Title: ANTIBODIES TO PLASMINOGEN ACTIVATOR INHIBITOR-1 (PAI-1) AND USES THEREOF. Applicant: Sanofi. Application EP14761451.5. The sequence listing filed with the application follows.

SEQUENCE LISTING (170 sequences)

SEQ ID NO: 1 - protein, 379 aa, Homo sapiens [sequence omitted]

SEQ ID NO: 2 - protein, 124 aa, Artificial Sequence
  mA105 VH
QVQLQQSGAELMKPGASVKISCKATGFTFSIYWIEWVKQRPGLGLEWIGEILPGSGSTNYNEKFKGKATFTADTSSNTAFMQLSSLTSEDSAVYYCARGGLYYDLDYWGQGTILTVSSAKTTPP

SEQ ID NO: 3 - protein, 115 aa, Artificial Sequence
  mA105 VL
DVVMTQTPLTLSVTIGQPASISCKSSQSLLDSDGKTYLNWLLQRPGQSPQRLISLVSKLDSGVPDRFTGSGSGTDFTLKLSRVEGADLGVYYCWQDRHFPRTFGGGTKLEIKRAD

SEQ ID NO: 4 - protein, 125 aa, Artificial Sequence
  mA39 VH
QVQLQQSGAELMKPGASVKISCKATGYTFNIYWIQWVKQRPGHGLEWIGEILPGSNTNYNEKFKDKATFTADSSSNTAYMQLSSLTSEDSAVYYCARLGIGLRGALDYWGQGTSVTVSSAKTTPP

SEQ ID NO: 5 - protein, 110 aa, Artificial Sequence
  mA39 VL
DIQMTHSPASLSASVGETVTITCRASENIYSYLAWYHQKQGKSPQLLVYNAKTLAEGVPSRFSGSGSGTQFSLNIKSLQPEDFGTFYCQHRYGSPWTFGGGTKLEIKRAD

SEQ ID NO: 6 - protein, 125 aa, Artificial Sequence
  mA44 VH
EMQLQESGPSLVKPSQTLSLTCSVTGDSMTNGYWNWIRKFPGNKLEYMGYITYSGSTYYNPSLKGRISITRNTSKNQYYLQLSSVTTEDTATYYCARWHYGSPYYFDYWGQGTTLTVSSAKTTPP

SEQ ID NO: 7 - protein, 110 aa, Artificial Sequence
  mA44 VL
DIKMTQSPSSMYASLGERVTITCKASQDINSYLSWLQQKPGKSPKTLIYRANRSVDGVPSRFSGSGSGQDYSLTISSLEYEDMGIYYCLQYDEFPPTFGGGTKLEIKRAD

SEQ ID NO: 8 - protein, 124 aa, Artificial Sequence
  mA71 VH
QVQLQQSGAELMKPGASVKISCKATGFTFSTYWIEWIKQRPGHGLDWIGEILPGSGNTNYNEKFKGKATFTADTSSNTVYMQLSSLTSEDSAVYYCARGGLYYNLDSWGQGTTLTVSSAKTTPP

SEQ ID NO: 9 - protein, 115 aa, Artificial Sequence
  mA71 VL
DVVMTQTPLTLSVTIGQPASISCKSSQSLLDSDGKTYLYWLLQRPGQSPKRLIYLVSKLDSGVPDRFTGSGSGTDFTLKISRVEAEDLGVYYCWQDTHFPRTFGGGTKLEIKRAD

SEQ ID NO: 10 - protein, 140 aa, Artificial Sequence
  mB109 VH
EVQLQQSGSVLARPGTSVKMSCKASGYSFTSYWMHWVKQRPGQGLEWMGAIYPGNSGQGLDWIGAIYPGNSDTTYNQKFEDKAKLTAVASASTAYMEVSSLTNEDSAVYYCTRGLRRWGAMDYWGQGTSVTVSSAKTTPP

SEQ ID NO: 11 - protein, 110 aa, Artificial Sequence
  mB109 VL
DIVMTQSHKFMSTSAGDRVSIPCKASQDVSSAVAWYQQKLGQSPKLLIYSASFRYTGVPDRFTGSGSGTDFTFTISSVQAEDLAVYYCQQHYSSPYTFGGGTNLEIKRAD

SEQ ID NO: 12 - protein, 125 aa, Artificial Sequence
  mB28 VH
QVQLQQSGAELMKPGASVKISCKATGYTFSISWIEWIKQRPGGLEWIGKILPGSGGANYNEKFKGKATVTADTSSNTVYMQLSSLTSEDSAVYYCARLSTGTRGAFDYWGQGTTLTVSSAKTTPP

SEQ ID NO: 13 - protein, 110 aa, Artificial Sequence
  mB28 VL
DIQLTQSPASLSASVGATVTITCRASENVYSYLAWYQQKQGKSPQLLVYNAKTLAEGVPSRFSGSGSGTQFSLKINYLQPEDFGSYYCQHHYGTPPTFGGGTKVEIKRAD

SEQ ID NO: 14 - protein, 121 aa, Artificial Sequence
  mC45 VH
QVQLQQSGVELVRPGTSVKVSCKASGYAFTNYLIEWIKQRPGQGLEWIGVIHPGSGVTNYNEKFKGKAILTADKSSSTAYMQLSSLTSDDSAVYFCARDYYGSSHGLMDYWGQGTSVTVSS

SEQ ID NO: 15 - protein, 107 aa, Artificial Sequence
  mC45 VL
DIKMTQSPSSMYASLGERVTITCKASQDINSYLSWFQQKPGKSPKTLIYRANRLVDGVPSRFSGSGSGQDYSLTISSLEYEDMGIYYCLQYDEFPRTFGGGTKLEIK

SEQ ID NO: 16 - protein, 118 aa, Artificial Sequence
  mE16 VH
EVKLVESGGGLVKPGGSLKLSCAASGFTFSNYGMSWVRQTPEKGLGWVASLRTGGNTYYSDSVKGRFTISRDNDRNILYLQMSSLTSEDTAVYYCARGLRHWGYFDVWGAGTTVTVSS

SEQ ID NO: 17 - protein, 107 aa, Artificial Sequence
  mE16 VL
DIVMTQSHKFMSTSVGDRVNITCKASQDVSTAVGWYQQEPGQSPKLLIYSASNRHTGVPDRFTGSGSGTDFTFTISSVQAEDLAVYYCQQHYSSPWTFGGGTKLEIK

SEQ ID NO: 18 - protein, 118 aa, Artificial Sequence
  mE21 VH
EVQLQQSGAELVRSGASVKLSCTASGFNIKDYYMHWVKQRPEQGLEWIGWIDPENGDTEYDPKFQAKATMTADTSSNTAYLQLSSLTSEDTAVYYCMYGNYPYYFDYWGQGTTLTVSS

SEQ ID NO: 19 - protein, 107 aa, Artificial Sequence
  mE21 VL
DIQMTQTTSSLSASLGDRVTISCRASQDISNYLNWYQQKPDGTVKLLIYYTSRLHSGVPSRFSGSGSGTDYSLTISNLEQEDIATYFCQQGNTLPWTFGGGTKLEIK

SEQ ID NO: 20 - protein, 11 aa, Artificial Sequence
  mA105 HCDR3
ARGGLYYDLDY

SEQ ID NO: 21 - protein, 8 aa, Artificial Sequence
  mA105 HCDR2
ILPGSGST

SEQ ID NO: 22 - protein, 8 aa, Artificial Sequence
  mA105 HCDR1
GFTFSIYW

SEQ ID NO: 23 - protein, 9 aa, Artificial Sequence
  mA105 LCDR3
WQDRHFPRT

SEQ ID NO: 24 - protein, 3 aa, Artificial Sequence
  mA105 LCDR2
LVS

SEQ ID NO: 25 - protein, 11 aa, Artificial Sequence
  mA105 LCDR1
QSLLDSDGKTY

SEQ ID NO: 26 - protein, 13 aa, Artificial Sequence
  mA39 HCDR3
ARLGIGLRGALDY

SEQ ID NO: 27 - protein, 7 aa, Artificial Sequence
  mA39 HCDR2
ILPGSNT

SEQ ID NO: 28 - protein, 8 aa, Artificial Sequence
  mA39 HCDR1
GYTFNIYW

SEQ ID NO: 29 - protein, 9 aa, Artificial Sequence
  mA39 LCDR3
QHRYGSPWT

SEQ ID NO: 30 - protein, 3 aa, Artificial Sequence
  mA39 LCDR2
NAK

SEQ ID NO: 31 - protein, 6 aa, Artificial Sequence
  mA38 LCDR1
ENIYSY

SEQ ID NO: 32 - protein, 13 aa, Artificial Sequence
  mA44 HCDR3
ARWHYGSPYYFDY

SEQ ID NO: 33 - protein, 7 aa, Artificial Sequence
  mA44 HCDR2
ITYSGST

SEQ ID NO: 34 - protein, 8 aa, Artificial Sequence
  mA44 HCDR1
GDSMTNGY

SEQ ID NO: 35 - protein, 9 aa, Artificial Sequence
  mA44 LCDR3
LQYDEFPPT

SEQ ID NO: 36 - protein, 3 aa, Artificial Sequence
  mA44 LCDR2
RAN

SEQ ID NO: 37 - protein, 6 aa, Artificial Sequence
  mA44 LCDR1
QDINSY

SEQ ID NO: 38 - protein, 11 aa, Artificial Sequence
  mA71 HCDR3
ARGGLYYNLDS

SEQ ID NO: 39 - protein, 8 aa, Artificial Sequence
  mA71 HCDR2
ILPGSGNT

SEQ ID NO: 40 - protein, 8 aa, Artificial Sequence
  mA71 HCDR1
GFTFSTYW

SEQ ID NO: 41 - protein, 9 aa, Artificial Sequence
  mA71 LCDR3
WQDTHFPRT

SEQ ID NO: 42 - protein, 3 aa, Artificial Sequence
  mA71 LCDR2
LVS

SEQ ID NO: 43 - protein, 11 aa, Artificial Sequence
  mA71 LCDR1
QSLLDSDGKTY

SEQ ID NO: 44 - protein, 11 aa, Artificial Sequence
  mA75 HCDR3
ARGGLYYAMDY

SEQ ID NO: 45 - protein, 8 aa, Artificial Sequence
  mA75 HCDR2
ILPGSGLT

SEQ ID NO: 46 - protein, 8 aa, Artificial Sequence
  mA75 HCDR1
GFTFSTYW

SEQ ID NO: 47 - protein, 9 aa, Artificial Sequence
  mA75 LCDR3
WQGSHFPQT

SEQ ID NO: 48 - protein, 3 aa, Artificial Sequence
  mA75 LCDR2
LVC

SEQ ID NO: 49 - protein, 11 aa, Artificial Sequence
  mA75 LCDR1
QSLLDSEGKTY

SEQ ID NO: 50 - protein, 12 aa, Artificial Sequence
  mB109 HCDR3
TRGLRRWGAMDY

SEQ ID NO: 51 - protein, 8 aa, Artificial Sequence
  mB109 HCDR2
ILPGSGLT

SEQ ID NO: 52 - protein, 8 aa, Artificial Sequence
  mB109 HCDR1
GFTFSTYW

SEQ ID NO: 53 - protein, 9 aa, Artificial Sequence
  mB109 LCDR3
QQHYSSPYT

SEQ ID NO: 54 - protein, 3 aa, Artificial Sequence
  mB109 LCDR2
SAS

SEQ ID NO: 55 - protein, 6 aa, Artificial Sequence
  mB109 LCDR1
QDVSSA

SEQ ID NO: 56 - protein, 13 aa, Artificial Sequence
  mB28 HCDR3
ARLSTGTRGAFDY

SEQ ID NO: 57 - protein, 8 aa, Artificial Sequence
  mB28 HCDR2
ILPGSGGA

SEQ ID NO: 58 - protein, 8 aa, Artificial Sequence
  mB28 HCDR1
GYTFSISW

SEQ ID NO: 59 - protein, 9 aa, Artificial Sequence
  mB28 LCDR3
QHHYGTPPT

SEQ ID NO: 60 - protein, 3 aa, Artificial Sequence
  mB28 LCDR2
NAK

SEQ ID NO: 61 - protein, 6 aa, Artificial Sequence
  mB28 LCDR1
ENVYSY

SEQ ID NO: 62 - protein, 14 aa, Artificial Sequence
  mC45 HCDR3
ARDYYGSSHGLMDY

SEQ ID NO: 63 - protein, 8 aa, Artificial Sequence
  mC45 HCDR2
IHPGSGVT

SEQ ID NO: 64 - protein, 8 aa, Artificial Sequence
  mC45 HCDR1
GYAFTNYL

SEQ ID NO: 65 - protein, 9 aa, Artificial Sequence
  mC45 LCDR3
LQYDEFPRT

SEQ ID NO: 66 - protein, 3 aa, Artificial Sequence
  mC45 LCDR2
RAN

SEQ ID NO: 67 - protein, 6 aa, Artificial Sequence
  mC45 LCDR1
QDINSY

SEQ ID NO: 68 - protein, 12 aa, Artificial Sequence
  mE16 HCDR3
ARGLRHWGYFDV

SEQ ID NO: 69 - protein, 7 aa, Artificial Sequence
  mE16 HCDR2
LRTGGNT

SEQ ID NO: 70 - protein, 8 aa, Artificial Sequence
  mE16 HCDR1
GFTFSNYG

SEQ ID NO: 71 - protein, 9 aa, Artificial Sequence
  mE16 LCDR3
QQHYSSPWT

SEQ ID NO: 72 - protein, 3 aa, Artificial Sequence
  mE16 LCDR2
SAS

SEQ ID NO: 73 - protein, 6 aa, Artificial Sequence
  mE16 LCDR1
QDISNY

SEQ ID NO: 74 - protein, 11 aa, Artificial Sequence
  mE21 HCDR3
MYGNYPYYFDY

SEQ ID NO: 75 - protein, 8 aa, Artificial Sequence
  mE21 HCDR2
IDPENGDT

SEQ ID NO: 76 - protein, 8 aa, Artificial Sequence
  mE21 HCDR1
GFNIKDYY

SEQ ID NO: 77 - protein, 9 aa, Artificial Sequence
  mE21 LCDR3
QQGNTLPWT

SEQ ID NO: 78 - protein, 3 aa, Artificial Sequence
  mE21 LCDR2
YTS

SEQ ID NO: 79 - protein, 6 aa, Artificial Sequence
  mE21 LCDR1
QDISNY

SEQ ID NO: 80 - protein, 124 aa, Artificial Sequence
  mA75 VH
QGQLQQSGAELMKPGASVKISCKASGFTFSTYWIAWLKQRPGHGLEWIAEILPGSGLTNYNEIFRGKATFTADTSSNTAYMQLSSLTSEDSAVYYCARGGLYYAMDYWGQGTSVTVSSAKTTAP

SEQ ID NO: 81 - protein, 114 aa, Artificial Sequence
  mA75 VL
DVVMTQTPLTLSVTIGQPASICKSSQSLLDSEGKTYLNWLFQRPGQSPKRLIYLVCKLDCGVPDRFTGSGSGTDFTLKISRVEGEDLGVYYCWQGSHFPQTFGGGTKLEIKRAD

SEQ ID NO: 82 - protein, 119 aa, Artificial Sequence
  HC1a
EMTLKESGPTLVKPTQTLSLTCSVTGDSMTNGYWNWIRKFPGKALEYMGYITYSGSTYYNPSLKGRISITRNTSKNQYYLTLSSVTTVDTATYYCARWHYGSPYYFDYWGQGTTLTVSS

SEQ ID NO: 83 - protein, 119 aa, Artificial Sequence
  HC1b
EMQLQESGPGLVKPSETLSLTCSVTGDSMTNGYWNWIRKFPGKGLEYMGYITYSGSTYYNPSLKGRISITRNTSKNQYYLKLSSVTTADTATYYCARWHYGSPYYFDYWGQGTTLTVSS

SEQ ID NO: 84 - protein, 119 aa, Artificial Sequence
  HC2a
EMTLKESGPTLVKPTQTLSLTCSVTGESMTQGYWNWIRKFPGKALEYMGYITYSGSTYYNPSLKGRISITRQTSKNQYYLTLSSVTTVETATYYCARWHYGSPYYFDYWGQGTTLTVSS

SEQ ID NO: 85 - protein, 119 aa, Artificial Sequence
  HC2b
EMTLKESGPTLVKPTQTLSLTCSVTGDSMTQGYWNWIRKFPGKALEYMGYITYSGSTYYNPSLKGRISITRNTSKNQYYLTLSSVTTVDTATYYCARWHYGSPYYFDYWGQGTTLTVSS

SEQ ID NO: 86 - protein, 119 aa, Artificial Sequence
  HC3
QMTLKESGPTLVKPTQTLSLTCSVSGDSMTNGYWNWIRQFPGKALEYMGYITYSGSTYYNPSLKGRITITRDTSKNQYYLTLSSVTTVDTATYYCARWHYGSPYYFDYWGQGTTLTVSS

SEQ ID NO: 87 - protein, 119 aa, Artificial Sequence
  HC4
QMTLKESGPTLVKPTQTLSLTCSVSGESMTQGYWNWIRQFPGKALEYMGYITYSGSTYYNPSLKGRITITRQTSKNQYYLTLSSVTTVETATYYCARWHYGSPYYFDYWGQGTTLTVSS

SEQ ID NO: 88 - protein, 119 aa, Artificial Sequence
  HC5a
QVQLQESGPGLVKPSETLSLTCTVSGDSMTNGYWNWIRQPPGKGLEYMGYITYSGSTYYNPSLKSRITISRNTSKNQYSLKLSSVTAADTAVYYCARWHYGSPYYFDYWGQGTLVTVSS

SEQ ID NO: 89 - protein, 119 aa, Artificial Sequence
  HC5b
QMQLQESGPGLVKPSETLSLTCTVSGDSMTNGYWNWIRQPPGKGLEYMGYITYSGSTYYNPSLKSRITISRDTSKNQYSLKLSSVTAADTAVYYCARWHYGSPYYFDYWGQGTLVTVSS

SEQ ID NO: 90 - protein, 119 aa, Artificial Sequence
  HC5c
QMQLQQSGPGLVKPSQTLSLTCAISGDSMTNGYWNWIRQSPSRGLEYMGYITYSGSTYYAVSVKSRITINRDTSKNQYSLQLSSVTPEDTAVYYCARWHYGSPYYFDYWGQGTLVTVSS

SEQ ID NO: 91 - protein, 107 aa, Artificial Sequence
  LC1a
DIKMTQSPSSLSASVGDRVTITCKASQDINSYLSWLQQKPGKSPKTLIYRANRSVDGVPSRFSGSGSGQDYSLTISSLQPEDLGIYYCLQYDEFPPTFGGGTKLEIK

SEQ ID NO: 92 - protein, 107 aa, Artificial Sequence
  LC1b
DIKMTQSPSSVSVSPGQTVTITCKASQDINSYLSWLQQKPGQSPKTLIYRANRSVDGVPSRFSGSGSGQDYSLTISSLQAMDEGIYYCLQYDEFPPTFGGGTKLTIK

SEQ ID NO: 93 - protein, 107 aa, Artificial Sequence
  LC2
DIKMTQSPSSLSASVGDRVTITCKASQDINSYLSWLQQKPGKSPKTLIYRAQRSVEGVPSRFSGSGSGQDYSLTISSLQPEDLGIYYCLQYDEFPPTFGGGTKLEIK

SEQ ID NO: 94 - protein, 107 aa, Artificial Sequence
  LC3
DIKMTQSPSSLSASVGDRVTITCKASQDINSYLSWLQQKPGKSPKTLIYRANRSVDGVPSRFSGSGSGQDYSLTISSLQPEDLATYYCLQYDEFPPTFGGGTKLEIK

SEQ ID NO: 95 - protein, 107 aa, Artificial Sequence
  LC4
DIKMTQSPSSLSASVGDRVTITCKASQDINSYLSWLQQKPGKSPKTLIYRAQRSVEGVPSRFSGSGSGQDYSLTISSLQPEDLATYYCLQYDEFPPTFGGGTKLEIK

SEQ ID NO: 96 - protein, 107 aa, Artificial Sequence
  LC5a
DIQMTQSPSSLSASVGDRVTITCKASQDINSYLSWLQQKPGKAPKLLIYRANRSVDGVPSRFSGSGSGTDYTFTISSLQPEDIATYYCLQYDEFPPTFGGGTKVEIK

SEQ ID NO: 97 - protein, 107 aa, Artificial Sequence
  LC5b
DIQMTQSPSSLSASVGDRVTITCKASQDINSYLSWLQQKPGKAPKTLIYRANRSVDGVPSRFSGSGSGQDYTFTISSLQPEDIATYYCLQYDEFPPTFGGGTKVEIK

SEQ ID NO: 98 - protein, 107 aa, Artificial Sequence
  LC5c
EIVMTQSPATLSLSPGERATLSCKASQDINSYLSWLQQKPGQAPRTLIYRANRSVDGIPARFSGSGSGQDYTLTISSLEPEDFAVYYCLQYDEFPPTFGGGTKVEIK

SEQ ID NO: 99 - protein, 255 aa, Artificial Sequence
  CH
ASTKGPSVFPLAPSSKSTSGGTAALGCLVKDYFPEPVTVSWNSGALTSGVHTFPAVLQSSGLYSLSSVVTVPSSSLGTQTYICNVNHKPSNTKVDKKVEPKSCDKTHTCPPCPAPELLGGPSVFLFPPKPKDTLMISRTPEVTCVVVDVSHEDPEVKFNWYVDGVEVHNAKTKPREEQYNSTYRVVSVLTVLHQDWLNGKEYKCKVSNKALPAPIEKTISKAKGQPREPQVYTLPPSRDELTKNQVSLTCLVKGF

SEQ ID NO: 100 - protein, 107 aa, Artificial Sequence [sequence omitted]

SEQ ID NO: 101 - protein, 107 aa, Artificial Sequence
  vk1
DIQMTQSPSSLSASVGDRVTITCRASQSISSYLNWYQQKPGKAPKLLIYAASSLQSGVPSRFSGSGSGTDFTLTISSLQPEDLATYYCQQSYSTPPTFGQGTKVEIK

SEQ ID NO: 102 - protein, 106 aa, Artificial Sequence
  vlambda3
  misc_feature (22)..(22): Xaa can be any naturally occurring amino acid
  misc_feature (87)..(87): Xaa can be any naturally occurring amino acid
SYELTQPPSVSVSPGQTASITXSGDKLGDKYASWYQQKPGQSPVLVIYQDSKRPSGIPERFSGSNSGNTATLTISGTQAMDEADYYXQAWDSSAVVFGGGTKLTVL

SEQ ID NO: 103 - protein, 120 aa, Artificial Sequence
  vh2
QVTLKESGPTLVKPTQTLTLTCTFSGFSLSTSGVGVGWIRQPPGKALEWLARIDWDDDKYYSTSLKTRLTISKDTSKNQVVLTMTNMDPVDTATYYCARMGFTGTYFDYWGQGTLVTVSS

SEQ ID NO: 104 - protein, 118 aa, Artificial Sequence
  vh4
  misc_feature (22)..(22): Xaa can be any naturally occurring amino acid
  misc_feature (95)..(95): Xaa can be any naturally occurring amino acid
QVQLQESGPGLVKPSETLSLTXTVSGGSISSYYWSWIRQPPGKGLEWIGYIYYSGSTNYNPSLKSRVTISVDTSKNQFSLKLSSVTAADTAVYYXARGDSSGYYFDYWGQGTLVTVSS

SEQ ID NO: 105 - DNA, 21 bp, Artificial Sequence
  Heavy Chain 3'- Primer
tatgcaaggcttacaaccaca

SEQ ID NO: 106 - DNA, 24 bp, Artificial Sequence
  Light Chain 3'- Primer
ctcattcctgttgaagctcttgag

SEQ ID NO: 107 - protein, 107 aa, Artificial Sequence
  IGKV1-33-01_IGKJ4-01
DIQMTQSPSSLSASVGDRVTITCQASQDISNYLNWYQQKPGKAPKLLIYDASNLETGVPSRFSGSGSGTDFTFTISSLQPEDIATYYCQQYDNLPLTFGGGTKVEIK

SEQ ID NO: 108 - protein, 119 aa, Artificial Sequence
  IGHV4-59-02_IGHD6-13-01_IGHJ4-02
QVQLQESGPGLVKPSETLSLTCTVSGGSVSSYYWSWIRQPPGKGLEWIGYIYYSGSTNYNPSLKSRVTISVDTSKNQFSLKLSSVTAADTAVYYCARGYSSSWYYFDYWGQGTLVTVSS

SEQ ID NO: 109 - protein, 226 aa, Artificial Sequence
  A44-hv1LC1a x HC1a
DIKMTQSPSSLSASVGDRVTITCKASQDINSYLSWLQQKPGKSPKTLIYRANRSVDGVPSRFSGSGSGQDYSLTISSLQPEDLGIYYCLQYDEFPPTFGGGTKLEIKEMTLKESGPTLVKPTQTLSLTCSVTGDSMTNGYWNWIRKFPGKALEYMGYITYSGSTYYNPSLKGRISITRNTSKNQYYLTLSSVTTVDTATYYCARWHYGSPYYFDYWGQGTTLTVSS

SEQ ID NO: 110 - protein, 226 aa, Artificial Sequence
  A44-hv2LC1b x HC1b
DIKMTQSPSSVSVSPGQTVTITCKASQDINSYLSWLQQKPGQSPKTLIYRANRSVDGVPSRFSGSGSGQDYSLTISSLQAMDEGIYYCLQYDEFPPTFGGGTKLTIKEMQLQESGPGLVKPSETLSLTCSVTGDSMTNGYWNWIRKFPGKGLEYMGYITYSGSTYYNPSLKGRISITRNTSKNQYYLKLSSVTTADTATYYCARWHYGSPYYFDYWGQGTTLTVSS

SEQ ID NO: 111 - protein, 226 aa, Artificial Sequence
  A44-hv3LC2 x HC2a
DIKMTQSPSSLSASVGDRVTITCKASQDINSYLSWLQQKPGKSPKTLIYRAQRSVEGVPSRFSGSGSGQDYSLTISSLQPEDLGIYYCLQYDEFPPTFGGGTKLEIKEMTLKESGPTLVKPTQTLSLTCSVTGESMTQGYWNWIRKFPGKALEYMGYITYSGSTYYNPSLKGRISITRQTSKNQYYLTLSSVTTVETATYYCARWHYGSPYYFDYWGQGTTLTVSS

SEQ ID NO: 112 - protein, 226 aa, Artificial Sequence
  A44-hv4LC1a x HC2b
DIKMTQSPSSLSASVGDRVTITCKASQDINSYLSWLQQKPGKSPKTLIYRANRSVDGVPSRFSGSGSGQDYSLTISSLQPEDLGIYYCLQYDEFPPTFGGGTKLEIKEMTLKESGPTLVKPTQTLSLTCSVTGDSMTQGYWNWIRKFPGKALEYMGYITYSGSTYYNPSLKGRISITRNTSKNQYYLTLSSVTTVDTATYYCARWHYGSPYYFDYWGQGTTLTVSS

SEQ ID NO: 113 - protein, 226 aa, Artificial Sequence
  A44-hv5LC2 x HC2b
DIKMTQSPSSLSASVGDRVTITCKASQDINSYLSWLQQKPGKSPKTLIYRAQRSVEGVPSRFSGSGSGQDYSLTISSLQPEDLGIYYCLQYDEFPPTFGGGTKLEIKEMTLKESGPTLVKPTQTLSLTCSVTGDSMTQGYWNWIRKFPGKALEYMGYITYSGSTYYNPSLKGRISITRNTSKNQYYLTLSSVTTVDTATYYCARWHYGSPYYFDYWGQGTTLTVSS

SEQ ID NO: 114 - protein, 226 aa, Artificial Sequence
  A44-hv6LC3 x HC3
DIKMTQSPSSLSASVGDRVTITCKASQDINSYLSWLQQKPGKSPKTLIYRANRSVDGVPSRFSGSGSGQDYSLTISSLQPEDLATYYCLQYDEFPPTFGGGTKLEIKQMTLKESGPTLVKPTQTLSLTCSVSGDSMTNGYWNWIRQFPGKALEYMGYITYSGSTYYNPSLKGRITITRDTSKNQYYLTLSSVTTVDTATYYCARWHYGSPYYFDYWGQGTTLTVSS

SEQ ID NO: 115 - protein, 226 aa, Artificial Sequence
  A44-hv7LC4 x HC4
DIKMTQSPSSLSASVGDRVTITCKASQDINSYLSWLQQKPGKSPKTLIYRAQRSVEGVPSRFSGSGSGQDYSLTISSLQPEDLATYYCLQYDEFPPTFGGGTKLEIKQMTLKESGPTLVKPTQTLSLTCSVSGESMTQGYWNWIRQFPGKALEYMGYITYSGSTYYNPSLKGRITITRQTSKNQYYLTLSSVTTVETATYYCARWHYGSPYYFDYWGQGTTLTVSS

SEQ ID NO: 116 - protein, 226 aa, Artificial Sequence
  A44-hv8LC5a x HC5a
DIQMTQSPSSLSASVGDRVTITCKASQDINSYLSWLQQKPGKAPKLLIYRANRSVDGVPSRFSGSGSGTDYTFTISSLQPEDIATYYCLQYDEFPPTFGGGTKVEIKQVQLQESGPGLVKPSETLSLTCTVSGDSMTNGYWNWIRQPPGKGLEYMGYITYSGSTYYNPSLKSRITISRNTSKNQYSLKLSSVTAADTAVYYCARWHYGSPYYFDYWGQGTLVTVSS

SEQ ID NO: 117 - protein, 226 aa, Artificial Sequence
  A44-hv9LC5b x HC5b
DIQMTQSPSSLSASVGDRVTITCKASQDINSYLSWLQQKPGKAPKTLIYRANRSVDGVPSRFSGSGSGQDYTFTISSLQPEDIATYYCLQYDEFPPTFGGGTKVEIKQMQLQESGPGLVKPSETLSLTCTVSGDSMTNGYWNWIRQPPGKGLEYMGYITYSGSTYYNPSLKSRITISRDTSKNQYSLKLSSVTAADTAVYYCARWHYGSPYYFDYWGQGTLVTVSS

SEQ ID NO: 118 - protein, 226 aa, Artificial Sequence
  A44-hv10LC5c x HC5c
EIVMTQSPATLSLSPGERATLSCKASQDINSYLSWLQQKPGQAPRTLIYRANRSVDGIPARFSGSGSGQDYTLTISSLEPEDFAVYYCLQYDEFPPTFGGGTKVEIKQMQLQQSGPGLVKPSQTLSLTCAISGDSMTNGYWNWIRQSPSRGLEYMGYITYSGSTYYAVSVKSRITINRDTSKNQYSLQLSSVTPEDTAVYYCARWHYGSPYYFDYWGQGTLVTVSS

SEQ ID NO: 119 - protein, 226 aa, Artificial Sequence
  A44-hv11LC2 x HC3
DIKMTQSPSSLSASVGDRVTITCKASQDINSYLSWLQQKPGKSPKTLIYRAQRSVEGVPSRFSGSGSGQDYSLTISSLQPEDLGIYYCLQYDEFPPTFGGGTKLEIKQMTLKESGPTLVKPTQTLSLTCSVSGDSMTNGYWNWIRQFPGKALEYMGYITYSGSTYYNPSLKGRITITRDTSKNQYYLTLSSVTTVDTATYYCARWHYGSPYYFDYWGQGTTLTVSS

SEQ ID NO: 120 - protein, 226 aa, Artificial Sequence
  A44-hv12LC4 X HC3
DIKMTQSPSSLSASVGDRVTITCKASQDINSYLSWLQQKPGKSPKTLIYRAQRSVEGVPSRFSGSGSGQDYSLTISSLQPEDLATYYCLQYDEFPPTFGGGTKLEIKQMTLKESGPTLVKPTQTLSLTCSVSGDSMTNGYWNWIRQFPGKALEYMGYITYSGSTYYNPSLKGRITITRDTSKNQYYLTLSSVTTVDTATYYCARWHYGSPYYFDYWGQGTTLTVSS

SEQ ID NO: 121 - protein, 226 aa, Artificial Sequence
  A44-hv13LC2 x HC5b
DIKMTQSPSSLSASVGDRVTITCKASQDINSYLSWLQQKPGKSPKTLIYRAQRSVEGVPSRFSGSGSGQDYSLTISSLQPEDLGIYYCLQYDEFPPTFGGGTKLEIKQMQLQESGPGLVKPSETLSLTCTVSGDSMTNGYWNWIRQPPGKGLEYMGYITYSGSTYYNPSLKSRITISRDTSKNQYSLKLSSVTAADTAVYYCARWHYGSPYYFDYWGQGTLVTVSS

SEQ ID NO: 122 - protein, 226 aa, Artificial Sequence
  A44-hv14LC4 x HC5b
DIKMTQSPSSLSASVGDRVTITCKASQDINSYLSWLQQKPGKSPKTLIYRAQRSVEGVPSRFSGSGSGQDYSLTISSLQPEDLATYYCLQYDEFPPTFGGGTKLEIKQMQLQESGPGLVKPSETLSLTCTVSGDSMTNGYWNWIRQPPGKGLEYMGYITYSGSTYYNPSLKSRITISRDTSKNQYSLKLSSVTAADTAVYYCARWHYGSPYYFDYWGQGTLVTVSS

SEQ ID NO: 123 - DNA, 255 bp, Artificial Sequence
  HC1a
gagatgaccctgaaagagtccggccccaccctggtcaaacccacccagaccctgagcctgacctgcagcgtgaccggcgacagcatgaccaacggctactggaactggatccggaagttccccggcaaggccctcgagtacatgggctacatcacctacagcggcagcacctactacaaccccagcctgaagggccggatcagcatcacccggaacaccagcaagaaccagtactacctgaccctgtccagcgtg

SEQ ID NO: 124 - DNA, 255 bp, Artificial Sequence
  HC1b
gagatgcagctgcaggaaagcggccctggcctggtcaaacccagcgagacactgagcctgacctgcagcgtgaccggcgacagcatgaccaacggctactggaactggatccggaagttccccggcaagggcctcgagtacatgggctacatcacctacagcggcagcacctactacaaccccagcctgaagggccggatcagcatcacccggaacaccagcaagaaccagtactacctgaagctgtccagcgtg

SEQ ID NO: 125 - DNA, 255 bp, Artificial Sequence
  HC2a
gagatgaccctgaaagagtccggccccaccctggtcaaacccacccagaccctgagcctgacctgcagcgtgaccggcgagagcatgacccagggctactggaactggatccggaagttccccggcaaggccctcgagtacatgggctacatcacctacagcggcagcacctactacaaccccagcctgaagggccggatcagcatcacccggcagaccagcaagaaccagtactacctgaccctgtccagcgtg

SEQ ID NO: 126 - DNA, 255 bp, Artificial Sequence
  HC2b
gagatgaccctgaaagagtccggccccaccctggtcaaacccacccagaccctgagcctgacctgcagcgtgaccggcgacagcatgacccagggctactggaactggatccggaagttccccggcaaggccctcgagtacatgggctacatcacctacagcggcagcacctactacaaccccagcctgaagggccggatcagcatcacccggaacaccagcaagaaccagtactacctgaccctgtccagcgtg

SEQ ID NO: 127 - DNA, 255 bp, Artificial Sequence
  HC3
cagatgaccctgaaagagtccggccccaccctggtcaaacccacccagaccctgagcctgacctgcagcgtgtccggcgacagcatgaccaacggctactggaactggatccggcagttccccggcaaggccctcgagtacatgggctacatcacctacagcggcagcacctactacaaccccagcctgaagggccggatcaccatcacccgggacaccagcaagaaccagtactacctgaccctgagcagcgtg

SEQ ID NO: 128 - DNA, 255 bp, Artificial Sequence
  HC4
cagatgaccctgaaagagtccggccccaccctggtcaaacccacccagaccctgagcctgacctgcagcgtgtccggcgagagcatgacccagggctactggaactggatccggcagttccccggcaaggccctcgagtacatgggctacatcacctacagcggcagcacctactacaaccccagcctgaagggccggatcaccatcacccggcagaccagcaagaaccagtactacctgaccctgagcagcgtg

SEQ ID NO: 129 - DNA, 255 bp, Artificial Sequence
  HC5a
caggtgcagctgcaggaaagcggccctggcctggtcaaacccagcgagacactgagcctgacctgcaccgtgtccggcgacagcatgaccaacggctactggaactggatccggcagccccctggcaagggcctcgagtacatgggctacatcacctacagcggcagcacctactacaaccccagcctgaagtcccggatcaccatcagccggaacaccagcaagaaccagtacagcctgaagctgagcagcgtg

SEQ ID NO: 130 - DNA, 255 bp, Artificial Sequence
  HC5b
cagatgcagctgcaggaaagcggccctggcctggtcaaacccagcgagacactgagcctgacctgcaccgtgtccggcgacagcatgaccaacggctactggaactggatccggcagccccctggcaagggcctcgagtacatgggctacatcacctacagcggcagcacctactacaaccccagcctgaagtcccggatcaccatcagccgggacaccagcaagaaccagtacagcctgaagctgagcagcgtg

SEQ ID NO: 131 - DNA, 255 bp, Artificial Sequence
  HC5c
cagatgcagctgcagcagagcggccctggcctggtcaaacccagccagaccctgagcctgacctgcgccatcagcggcgacagcatgaccaacggctactggaactggatccggcagagccccagcagaggcctcgagtacatgggctacatcacctacagcggcagcacctactacgccgtgtccgtgaagtcccggatcaccatcaaccgggacaccagcaagaaccagtacagcctgcagctgagcagcgtg

SEQ ID NO: 132 - DNA, 255 bp, Artificial Sequence
  LC1a
gacatcaagatgacccagagccccagcagcctgagcgccagcgtgggcgacagagtgaccatcacatgcaaggccagccaggacatcaacagctacctgagctggctgcagcagaagcccggcaagagccccaagaccctgatctaccgggccaaccgcagcgtggacggcgtgccaagcagattttccggcagcggcagcggccaggactacagcctgaccatcagcagcctgcagcccgaggacctgggcatc

SEQ ID NO: 133 - DNA, 255 bp, Artificial Sequence
  LC1b
gacatcaagatgacccagagccccagcagcgtgtccgtgtctcctggccagaccgtgaccatcacatgcaaggccagccaggacatcaacagctacctgagctggctgcagcagaagcccggccagtcccccaagaccctgatctaccgggccaaccgcagcgtggacggcgtgccaagcagattttccggcagcggcagcggccaggactacagcctgaccatcagcagcctgcaggccatggacgagggcatc

SEQ ID NO: 134 - DNA, 255 bp, Artificial Sequence
  LC2
gacatcaagatgacccagagccccagcagcctgagcgccagcgtgggcgacagagtgaccatcacatgcaaggccagccaggacatcaacagctacctgagctggctgcagcagaagcccggcaagagccccaagaccctgatctaccgggcccagcggagcgtggaaggcgtgccaagcagattcagcggcagcggctccggccaggactacagcctgaccatcagcagcctgcagcccgaggacctgggcatc

SEQ ID NO: 135 - DNA, 255 bp, Artificial Sequence
  LC3
gacatcaagatgacccagagccccagcagcctgagcgccagcgtgggcgacagagtgaccatcacatgcaaggccagccaggacatcaacagctacctgagctggctgcagcagaagcccggcaagagccccaagaccctgatctaccgggccaaccgcagcgtggacggcgtgccaagcagattttccggcagcggcagcggccaggactacagcctgaccatcagcagcctgcagcccgaggacctggccacc

SEQ ID NO: 136 - DNA, 255 bp, Artificial Sequence
  LC4
gacatcaagatgacccagagccccagcagcctgagcgccagcgtgggcgacagagtgaccatcacatgcaaggccagccaggacatcaacagctacctgagctggctgcagcagaagcccggcaagagccccaagaccctgatctaccgggcccagcggagcgtggaaggcgtgccaagcagattcagcggcagcggctccggccaggactacagcctgaccatcagcagcctgcagcccgaggacctggccacc

SEQ ID NO: 137 - DNA, 255 bp, Artificial Sequence
  LC5a
gacatccagatgacccagagccccagcagcctgagcgccagcgtgggcgacagagtgaccatcacatgcaaggccagccaggacatcaacagctacctgagctggctgcagcagaagcccggcaaggcccccaagctgctgatctaccgggccaaccgcagcgtggacggcgtgccaagcagattttccggcagcggctccggcaccgactacaccttcaccatcagcagcctgcagcccgaggatatcgccacc

SEQ ID NO: 138 - DNA, 255 bp, Artificial Sequence
  LC5b
gacatccagatgacccagagccccagcagcctgagcgccagcgtgggcgacagagtgaccatcacatgcaaggccagccaggacatcaacagctacctgagctggctgcagcagaagcccggcaaggcccccaagaccctgatctaccgggccaaccgcagcgtggacggcgtgccaagcagattttccggcagcggcagcggccaggactacaccttcaccatcagcagcctgcagcccgaggatatcgccacc

SEQ ID NO: 139 - DNA, 255 bp, Artificial Sequence
  LC5c
gagatcgtgatgacccagagccccgccaccctgtctctgagccctggcgagagagccaccctgagctgcaaggccagccaggacatcaacagctacctgagctggctgcagcagaagcccggccaggcccccagaaccctgatctaccgggccaacagaagcgtggacggcatccccgccagattcagcggcagcggctccggccaggactacaccctgaccatcagcagcctggaacccgaggacttcgccgtg

SEQ ID NO: 140 - protein, 119 aa, Artificial Sequence
  mA44 VH
EMQLQESGPSLVKPSQTLSLTCSVTGDSMTNGYWNWIRKFPGNKLEYMGYITYSGSTYYNPSLKGRISITRNTSKNQYYLQLSSVTTEDTATYYCARWHYGSPYYFDYWGQGTTLTVSS

SEQ ID NO: 141 - protein, 107 aa, Artificial Sequence
  mA44 VL
DIKMTQSPSSMYASLGERVTITCKASQDINSYLSWLQQKPGKSPKTLIYRANRSVDGVPSRFSGSGSGQDYSLTISSLEYEDMGIYYCLQYDEFPPTFGGGTKLEIK

SEQ ID NO: 142 - protein, 118 aa, Artificial Sequence
  mA44 VL
DIKMTQSPSSMYASLGERVTITCKASQDINSYLSWLQQKPGKSPKTLIYRANRSVDGVPSRFSGSGSGQDYSLTISSLEYEDMGIYYCLQYDEFPPTFGGGTKLEIKRADAAPTVSIF

SEQ ID NO: 143 - protein, 107 aa, Artificial Sequence
  IGKV3-11-02_IGKJ4-0
EIVLTQSPATLSLSPGERATLSCRASQSVSSYLAWYQQKPGQAPRLLIYDASNRATGIPARFSGSGSGRDFTLTISSLEPEDFAVYYCQQRSNWPLTFGGGTKVEIK

SEQ ID NO: 144 - protein, 123 aa, Artificial Sequence
  IGHV6-1-02_IGHD6-13-01_IGHJ4-02
QVQLQQSGPGLVKPSQTLSLTCAISGDSVSSNSAAWNWIRQSPSRGLEWLGRTYYRSKWYNDYAVSVKSRITINPDTSKNQFSLQLNSVTPEDTAVYYCARGYSSSWYYFDYWGQGTLVTVSS

SEQ ID NO: 145 - protein, 3 aa, Artificial Sequence
  Synthetic
RAQ

SEQ ID NO: 146 - protein, 8 aa, Artificial Sequence
  Synthetic
GESMTQGY

SEQ ID NO: 147 - protein, 8 aa, Artificial Sequence
  Synthetic
GDSMTQGY

SEQ ID NO: 148 - protein, 117 aa, Artificial Sequence
  Synthetic
QVKLQESGPELVKPGASVKISCKASGYSFTDYNMNWVKQSKGKSLEWIGIIHPNSGTTTYNQKFKGKATLTVDQSSSTAYLQLNSLTSEDSAVYYCARSKLRFFDYWGQGTTVTVSS

SEQ ID NO: 149 - protein, 107 aa, Artificial Sequence
  Synthetic
DIKLTQSPSSMYASLGERVTITCKASQDIYSYLSWFQQKPGKSPKTLIYRANRLIDGVPSRFSGSGSGQDYSLTISSLEYEHMGIYYCLQYDEFPFTFGSGTKLEIK

SEQ ID NO: 150 - protein, 107 aa, Artificial Sequence
  Synthetic
DIQMTQSPSSLSASVGDRVTITCQASQDISNYLNWYQQKPGKAPKLLIYDASNLETGVPSRFSGSGSGTDFTFTISSLQPEDIATYYCQQYDNLPCSFGQGTKLEIK

SEQ ID NO: 151 - protein, 118 aa, Artificial Sequence
  Synthetic
  misc_feature (99)..(103): Xaa can be any naturally occurring amino acid
QVQLVQSGSELKKPGASVKVSCKASGYTFTSYAMNWVRQAPGQGLEWMGWINTNTGNPTYAQGFTGRFVFSLDTSVSTAYLQISSLKAEDTAVYYCARXXXXXYFDYWGQGTLVTVSS

SEQ ID NO: 152 - protein, 118 aa, Artificial Sequence
  Synthetic
  misc_feature (99)..(103): Xaa can be any naturally occurring amino acid
QVQLVQSGAEVKKPGASVKVSCKASGYTFTSYYMHWVRQAPGQGLEWMGIINPSGGSTSYAQKFQGRVTMTRDTSTSTVYMELSSLRSEDTAVYYCARXXXXXYFDYWGQGTLVTVSS

SEQ ID NO: 153 - protein, 107 aa, Artificial Sequence
  Synthetic
DIQLTQSPSSLSASVGDRVTITCKASQDIYSYLSWFQQKPGKAPKTLIYRANRLIDGVPSRFSGSGSGQDYTFTISSLQPEDIATYYCLQYDEFPFTFGQGTKLEIK

SEQ ID NO: 154 - protein, 117 aa, Artificial Sequence
  Synthetic
QVQLVQSGSELKKPGASVKVSCKASGYSFTDYNMNWVRQAPGQGLEWIGIIHPNSGTTTYNQKFKGRAVLSVDQSVSTAYLQISSLKAEDTAVYYCARSKLRFFDYWGQGTLVTVSS

SEQ ID NO: 155 - protein, 117 aa, Artificial Sequence
  Synthetic
QVQLVQSGAEVKKPGASVKVSCKASGYSFTDYNMNWVRQAPGQGLEWIGIIHPNSGTTTYNQKFKGRATLTVDQSTSTAYMELSSLRSEDTAVYYCARSKLRFFDYWGQGTLVTVSS

SEQ ID NO: 156 - protein, 4 aa, Artificial Sequence
  Synthetic
  misc_feature (2)..(3): Xaa can be any naturally occurring amino acid
EXXQ

SEQ ID NO: 157 - protein, 3 aa, Artificial Sequence
  Synthetic
  misc_feature (2)..(2): Xaa can be any naturally occurring amino acid
LXR

SEQ ID NO: 158 - protein, 20 aa, Artificial Sequence
  Synthetic
  misc_feature (3)..(4): Xaa can be any naturally occurring amino acid
  misc_feature (13)..(14): Xaa can be any naturally occurring amino acid
TDXXRQFQADFTXXSDQEPL

SEQ ID NO: 159 - protein, 11 aa, Artificial Sequence
  Artificial Sequence
TTGGETRQQIQ

SEQ ID NO: 160 - protein, 3 aa, Artificial Sequence
  Artificial Sequence
RHL

SEQ ID NO: 161 - protein, 22 aa, Artificial Sequence
  Artificial Sequence
  misc_feature (4)..(6): Xaa can be any naturally occurring amino acid
TDMXXXFQADFTSLSNQEPLHV

SEQ ID NO: 162 - protein, 402 aa, cynomolgus
MQMSPALACLVLGLAFVFGEGSTVHHPPSYVAHLASDFGVRVFQQVAQASKDRNVVFSPYGVASVLAMLQLTTGGETRQQIQAAMGFKIDDKGMAPALRHLYKELLGPWNKDEISTTDAIFVQRDLKLVQGFMPHFFRLFRSTVKQVDFSEAERARFIINDWVKTHTKGMISDLLGKGAVDQLTRLVLVNALYFNGHWKTPFPDSSTHRRLFHKSDGSTVSVPMMAQTNKFNYTEFTTPDGHYYDILELPYHGNTLSMFIAAPYEKQVPLSALTNILSAQLISHWKGNMTRLPRLLVLPKFSLETEVDLRKPLENLGMTDMFRQFQADFTSLSNQEPLHVAQALQKVKIEVNESGTVASSSTAVIVSARMAPEEIIMDRPFLFVVRHNPTGTVLFMGQVMEP

SEQ ID NO: 163 - protein, 402 aa, Mus musculus
MQMSSALACLILGLVLVSGKGFTLPLRESHTAHQATDFGVKVFQQVVQASKDRNVVFSPYGVSSVLAMLQMTTAGKTRRQIQDAMGFKVNEKGTAHALRQLSKELMGPWNKNEISTADAIFVQRDLELVQGFMPHFFKLFQTMVKQVDFSEVERARFIINDWVERHTKGMISDLLAKGAVDELTRLVLVNALYFSGQWKTPFLEASTHQRLFHKSDGSTVSVPMMAQSNKFNYTEFTTPDGLEYDVVELPYQGDTLSMFIAAPFEKDVHLSALTNILDAELIRQWKGNMTRLPRLLILPKFSLETEVDLRGPLEKLGMPDMFSATLADFTSLSDQEQLSVAQALQKVRIEVNESGTVASSSTAFVISARMAPTEMVIDRSFLFVVRHNPTETILFMGQVMEP

SEQ ID NO: 164 - protein, 402 aa, Rattus norvegicus
MQMSSALTCLTLGLVLVFGKGFASPLPESHTAQQATNFGVKVFQHVVQASKDRNVVFSPYGVSSVLAMLQLTTAGKTRQQIQDAMGFNISERGTAPALRKLSKELMGSWNKNEISTADAIFVQRDLELVQGFMPHFFKLFRTTVKQVDFSEVERARFIINDWVERHTKGMISDLLAKGAVNELTRLVLVNALYFNGQWKTPFLEASTHQRLFHKSDGSTISVPMMAQNNKFNYTEFTTPDGHEYDILELPYHGETLSMFIAAPFEKDVPLSAITNILDAELIRQWKSNMTRLPRLLILPKFSLETEVDLRGPLEKLGMTDIFSSTQADFTSLSDQEQLSVAQALQKVKIEVNESGTVASSSTAILVSARMAPTEMVLDRSFLFVVRHNPTETILFMGQLMEP

SEQ ID NO: 165 - protein, 6 aa, Artificial Sequence
  Synthetic
QDIYSY

SEQ ID NO: 166 - protein, 9 aa, Artificial Sequence
  Synthetic
LQYDEFPFT

SEQ ID NO: 167 - protein, 3 aa, Artificial Sequence
  Synthetic
RAN

SEQ ID NO: 168 - protein, 8 aa, Artificial Sequence
  Synthetic
GYSFTDYN

SEQ ID NO: 169 - protein, 9 aa, Artificial Sequence
  Synthetic
LQYDEFPFT

SEQ ID NO: 170 - protein, 3 aa, Artificial Sequence
  Synthetic
RAN